European Patent Application EP 4 450 093 A1, published October 23, 2024. Title: Cleavable Immune Cell Engagers. Applicant: Synaffix B.V. The sequence listing filed with the application follows.

SEQUENCE LISTING (26 sequences)

SEQ ID NO: 1 - protein, 26 aa, synthetic construct
  source 1..26: note = protease-cleavable linker 1
GSSGGSGGSGGSGLSGRSDNHGSSGS

SEQ ID NO: 2 - protein, 18 aa, synthetic construct
  source 1..18: note = protease-cleavable linker 2
GGGGSGGGGSRASRANGS

SEQ ID NO: 3 - protein, 114 aa, Homo sapiens
  source 1..114: note = human IL-15
NWVNVISDLKKIEDLIQSMHIDATLYTESDVHPSCKVTAMKCFLLELQVISLESGDASIHDTVENLIILANNSLSSNGNVTESGCKECEELEEKNIKEFLQSFVHIVQMFINTS

SEQ ID NO: 4 - protein, 211 aa, synthetic construct
  source 1..211: note = IL-15Ra-IL-15 fusion protein
ITCPPPMSVEHADIWVKSYSLYSRERYICNSGFKRKAGTSSLTECVLNKATNVAHWTTPSLKCIRDPALVHQRPAPPSGGSGGGGSGGGSGGGGSLQNWVNVISDLKKIEDLIQSMHIDATLYTESDVHPSCKVTAMKCFLLELQVISLESGDASIHDTVENLIILANNSLSSNGNVTESGCKECEELEEKNIKEFLQSFVHIVQMFINTS

SEQ ID NO: 5 - protein, 132 aa, synthetic construct
  source 1..132: note = SYR-(G4S)3-IL15 (PF18)
SYRGGGGSGGGGSGGGGSNWVNVISDLKKIEDLIQSMHIDATLYTESDVHPSCKVTAMKCFLLELQVISLESGDASIHDTVENLIILANNSLSSNGNVTESGCKECEELEEKNIKEFLQSFVHIVQMFINTS

SEQ ID NO: 6 - protein, 144 aa, synthetic construct
  source 1..144: note = SYR-cleavable linker 1-IL15 (PF50)
MSYRGSSGGSGGSGGSGLSGRSDNHGSSGSNWVNVISDLKKIEDLIQSMHIDATLYTESDVHPSCKVTAMKCFLLELQVISLESGDASIHDTVENLIILANNSLSSNGNVTESGCKECEELEEKNIKEFLQSFVHIVQMFINTS

SEQ ID NO: 7 - protein, 136 aa, synthetic construct
  source 1..136: note = SYR-cleavable linker 2-IL15 (PF51)
MSYRGGGGSGGGGSRASRANGSNWVNVISDLKKIEDLIQSMHIDATLYTESDVHPSCKVTAMKCFLLELQVISLESGDASIHDTVENLIILANNSLSSNGNVTESGCKECEELEEKNIKEFLQSFVHIVQMFINTS

SEQ ID NO: 8 - protein, 134 aa, synthetic construct
  source 1..134: note = ST-cleavable linker 2-IL15 (PF52)
STGGGGSGGGGSRASRANGSNWVNVISDLKKIEDLIQSMHIDATLYTESDVHPSCKVTAMKCFLLELQVISLESGDASIHDTVENLIILANNSLSSNGNVTESGCKECEELEEKNIKEFLQSFVHIVQMFINTS

SEQ ID NO: 9 - protein, 134 aa, synthetic construct
  source 1..134: note = ST-cleavable linker 2-IL15(N72D) (PF53)
STGGGGSGGGGSRASRANGSNWVNVISDLKKIEDLIQSMHIDATLYTESDVHPSCKVTAMKCFLLELQVISLESGDASIHDTVENLIILANDSLSSNGNVTESGCKECEELEEKNIKEFLQSFVHIVQMFINTS

SEQ ID NO: 10 - protein, 134 aa, synthetic construct
  source 1..134: note = ST-(G4S)3GGS-IL15 (PF54)
STGGGGSGGGGSGGGGSGGSNWVNVISDLKKIEDLIQSMHIDATLYTESDVHPSCKVTAMKCFLLELQVISLESGDASIHDTVENLIILANNSLSSNGNVTESGCKECEELEEKNIKEFLQSFVHIVQMFINTS

SEQ ID NO: 11 - protein, 157 aa, synthetic construct
  source 1..157: note = SYR-(G4S)8-IL15 (PF55)
SYRGGGGSGGGGSGGGGSGGGGSGGGGSGGGGSGGGGSGGGGSNWVNVISDLKKIEDLIQSMHIDATLYTESDVHPSCKVTAMKCFLLELQVISLESGDASIHDTVENLIILANNSLSSNGNVTESGCKECEELEEKNIKEFLQSFVHIVQMFINTS

SEQ ID NO: 12 - protein, 135 aa, synthetic construct
  source 1..135: note = ST-cleavable linker 2-IL15(E46G,V49R) (PF56)
MSTGGGGSGGGGSRASRANGSNWVNVISDLKKIEDLIQSMHIDATLYTESDVHPSCKVTAMKCFLLGLQRISLESGDASIHDTVENLIILANNSLSSNGNVTESGCKECEELEEKNIKEFLQSFVHIVQMFINTS

SEQ ID NO: 13 - protein, 255 aa, synthetic construct
  source 1..255: note = SYR-(G4S)8-IL15Ra-IL-15 (PF57)
MSYRGGGGSGGGGSGGGGSGGGGSGGGGSGGGGSGGGGSGGGGSITCPPPMSVEHADIWVKSYSLYSRERYICNSGFKRKAGTSSLTECVLNKATNVAHWTTPSLKCIRDPALVHQRPAPPSGGSGGGGSGGGSGGGGSLQNWVNVISDLKKIEDLIQSMHIDATLYTESDVHPSCKVTAMKCFLLELQVISLESGDASIHDTVENLIILANNSLSSNGNVTESGCKECEELEEKNIKEFLQSFVHIVQMFINTS

SEQ ID NO: 14 - protein, 252 aa, synthetic construct
  source 1..252: note = S-(G4S)8-IL15Ra-IL-15 (PF58)
SGGGGSGGGGSGGGGSGGGGSGGGGSGGGGSGGGGSGGGGSITCPPPMSVEHADIWVKSYSLYSRERYICNSGFKRKAGTSSLTECVLNKATNVAHWTTPSLKCIRDPALVHQRPAPPSGGSGGGGSGGGSGGGGSLQNWVNVISDLKKIEDLIQSMHIDATLYTESDVHPSCKVTAMKCFLLELQVISLESGDASIHDTVENLIILANNSLSSNGNVTESGCKECEELEEKNIKEFLQSFVHIVQMFINTS

SEQ ID NO: 15 - protein, 253 aa, synthetic construct
  source 1..253: note = ST-(G4S)8-IL15Ra-IL-15 (PF59)
STGGGGSGGGGSGGGGSGGGGSGGGGSGGGGSGGGGSGGGGSITCPPPMSVEHADIWVKSYSLYSRERYICNSGFKRKAGTSSLTECVLNKATNVAHWTTPSLKCIRDPALVHQRPAPPSGGSGGGGSGGGSGGGGSLQNWVNVISDLKKIEDLIQSMHIDATLYTESDVHPSCKVTAMKCFLLELQVISLESGDASIHDTVENLIILANNSLSSNGNVTESGCKECEELEEKNIKEFLQSFVHIVQMFINTS

SEQ ID NO: 16 - protein, 215 aa, synthetic construct
  source 1..215: note = mPD-L1 light chain
QSALTQPASVSGSPGQSITISCTGTSSDVGAYNYVSWYQQHPGKAPKLMIYDVSNRPSGVSNRFSGSKSGNTASLTISGLQAEDEADYYCSSYTSSSTRVFGTGTKVTVLGQPKANPTVTLFPPSSEELQANKATLVCLISDFYPGAVTVAWKADGSPVKAGVETTKPSKQSNNKYAASSYLSLTPEQWKSHRSYSCQVTHEGSTVEKTVAPTEC

SEQ ID NO: 17 - protein, 450 aa, synthetic construct
  source 1..450: note = mPD-L1 heavy chain
EVQLLESGGGLVQPGGSLRLSCAASGFTFSAYRMFWVRQAPGKGLEWVSSIYPSGGITFYADSVKGRFTISRDNSKNTLYLQMNSLRAEDTAIYYCARIKLGTVTTVDYWGQGTLVTVSSASTKGPSVFPLAPSSKSTSGGTAALGCLVKDYFPEPVTVSWNSGALTSGVHTFPAVLQSSGLYSLSSVVTVPSSSLGTQTYICNVNHKPSNTKVDKRVEPKSCDKTHTCPPCPAPELLGGPSVFLFPPKPKDTLMISRTPEVTCVVVDVSHEDPEVKFNWYVDGVEVHNAKTKPREEQYNSTYRVVSVLTVLHQDWLNGKEYKCKVSNKALPAPIEKTISKAKGQPREPQVYTLPPSREEMTKNQVSLTCLVKGFYPSDIAVEWESNGQPENNYKTTPPVLDSDGSFFLYSKLTVDKSRWQQGNVFSCSVMHEALHNHYTQKSLSLSPGK

SEQ ID NO: 18 - protein, 659 aa, synthetic construct
  source 1..659: note = genetic fusion (IC1) heavy chain
EVQLLESGGGLVQPGGSLRLSCAASGFTFSAYRMFWVRQAPGKGLEWVSSIYPSGGITFYADSVKGRFTISRDNSKNTLYLQMNSLRAEDTAIYYCARIKLGTVTTVDYWGQGTLVTVSSASTKGPSVFPLAPSSKSTSGGTAALGCLVKDYFPEPVTVSWNSGALTSGVHTFPAVLQSSGLYSLSSVVTVPSSSLGTQTYICNVNHKPSNTKVDKRVEPKSCDKTHTCPPCPAPEAAGGPSVFLFPPKPKDTLMISRTPEVTCVVVDVSHEDPEVKFNWYVDGVEVHNAKTKPREEQYNSTYRVVSVLTVLHQDWLNGKEYKCKVSNKALPAPIEKTISKAKGQPREPQVYTLPPSREEMTKNQVSLTCLVKGFYPSDIAVEWESNGQPENNYKTTPPVLDSDGSFFLYSKLTVDKSRWQQGNVFSCSVMHEALHNHYTQKSLSLSPGSCPPPMSVEHADIWVKSYSLYSRERYICNSGFKRKAGTSSLTECVLNKATNVAHWTTPSLKCIRDPALVHQRPAPPSGGSGGGGSGGGSGGGGSLQNWVNVISDLKKIEDLIQSMHIDATLYTESDVHPSCKVTAMKCFLLELQVISLESGDASIHDTVENLIILANNSLSSNGNVTESGCKECEELEEKNIKEFLQSFVHIVQMFINTS

SEQ ID NO: 19 - protein, 4 aa, synthetic construct
  source 1..4: note = peptide spacer 1
GGGG

SEQ ID NO: 20 - protein, 4 aa, synthetic construct
  source 1..4: note = peptide spacer 2
GGFG

SEQ ID NO: 21 - protein, 4 aa, synthetic construct
  source 1..4: note = peptide spacer 3
GFGG

SEQ ID NO: 22 - protein, 4 aa, synthetic construct
  source 1..4: note = peptide spacer 4
FGGG

SEQ ID NO: 23 - protein, 4 aa, synthetic construct
  source 1..4: note = peptide spacer 5
GGGF

SEQ ID NO: 24 - protein, 4 aa, synthetic construct
  source 1..4: note = peptide spacer 6
FFGG

SEQ ID NO: 25 - protein, 4 aa, synthetic construct
  source 1..4: note = peptide spacer 7
GGFF

SEQ ID NO: 26 - protein, 5 aa, synthetic construct
  source 1..5: note = peptide spacer 8
GGGFG